European Patent Specification EP 3 950 126 B1, published June 24, 2026. Title: Inorganic porous carrier and method of producing nucleic acid using the same. Applicant: SUMITOMO CHEMICAL COMPANY, LIMITED. The sequence listing filed with the application follows.

SEQUENCE LISTING (3 sequences)

SEQ ID NO: 1 - RNA, 23 nt, Artificial Sequence
  Synthesized RNA
gcagaguacacacagcauauacc

SEQ ID NO: 2 - RNA, 25 nt, Artificial Sequence
  Synthesized RNA
gguauaugcuguguguacucugcuu

SEQ ID NO: 3 - RNA, 103 nt, Artificial Sequence
  Syntesized RNA
auaacucaauuuguaaaaaaguuuuagagcuagaaauagcaaguuaaaauaaggcuaguccguuaucaacuugaaaaaguggcaccgagucggugcuuuuuuu